European Patent Application EP 4 806 996 A1, published September 16, 2026. Title: 新型Endo S2突变体酶. Applicant: 上海齐鲁制药研究中心有限公司. Application CN. The sequence listing filed with the application follows.

SEQUENCE LISTING (1 sequence)

SEQ ID NO: 1 - protein, 843 aa, Streptococcus pyogenes
MDKHLLVKRTLGCVCAATLMGAALATHHDSLNTVKAEEKTVQTGKTDQQVGAKLVQEIREGKRGPLYAGYFRTWHDRASTGIDGKQQHPENTMAEVPKEVDILFVFHDHTASDSPFWSELKDSYVHKLHQQGTALVQTIGVNELNGRTGLSKDYPDTPEGNKALAAAIVKAFVTDRGVDGLDIDIEHEFTNKRTPEEDARALNVFKEIAQLIGKNGSDKSKLLIMDTTLSVENNPIFKGIAEDLDYLLRQYYGSQGGEAEVDTINSDWNQYQNYIDASQFMIGFSFFEESASKGNLWFDVNEYDPNNPEKGKDIEGTRAKKYAEWQPSTGGLKAGIFSYAIDRDGVAHVPSTYKNRTSTNLQRHEVDNISHTDYTVSRKLKTLMTEDKRYDVIDQKDIPDPALREQIIQQVGQYKGDLERYNKTLVLTGDKIQNLKGLEKLSKLQKLELRQLSNVKEITPELLPESMKKDAELVMVGMTGLEKLNLSGLNRQTLDGIDVNSITHLTSFDISHNSLDLSEKSEDRKLLMTLMEQVSNHQKITVKNTAFENQKPKGYYPQTYDTKEGHYDVDNAEHDILTDFVFGTVTKRNTFIGDEEAFAIYKEGAVDGRQYVSKDYTYEAFRKDYKGYKVHLTASNLGETVTSKVTATTDETYLVDVSDGEKVVHHMKLNIGSGAIMMENLAKGAKVIGTSGDFEQAKKIFDGEKSDRFFTWGQTNWIAFDLGEINLAKEWRLFNAETNTEIKTDSSLNVAKGRLQILKDTTIDLEKMDIKNRKEYLSNDENWTDVAQMDDAKAIFNSKLSNVLSRYWRFCVDGGASSYYPQYTELQILGQRLSNDVANTLKD